European Patent Application EP 4 553 164 A2, published May 14, 2025. Title: 经修饰的自复制mRNA. Applicant: 嘉晨西海（杭州）生物技术有限公司. Application CN. The sequence listing filed with the application follows.

SEQUENCE LISTING (3 sequences)

SEQ ID NO: 1 - DNA, 750 bp, synthetic construct
  source 1..750: mol_type = other DNA
atgcccatggggtctctgcaaccgctggccaccttgtacctgctggggatgctggtcgcttccgtgctagcctctagacgggtgcagcctacagagagcatcgtgcggttccctaacatcaccaacctctgccccttcggcgaggtgttcaacgccaccagattcgccagcgtctacgcctggaaccggaagcggatcagcaattgcgtggccgactacagcgtgctgtacaacagcgccagcttcagcaccttcaagtgctacggcgtgtcccctaccaagctgaacgatctgtgcttcaccaacgtgtacgccgacagcttcgtgatcaggggcgacgaagtgcgacagatcgccccaggacagacaggaaagatcgccgattacaactacaagctgcccgacgacttcaccggttgcgtgatcgcttggaacagcaacaacctggacagcaaggtcggcggcaactacaactacctgtaccggctgttccggaagtccaacctgaagcccttcgagcgggacatcagcacagagatctaccaggccggcagcacaccttgtaacggcgtggagggcttcaactgctacttccctctgcagagctacggcttccagcctacaaacggcgtgggataccagccttacagggtggtggtgctgagcttcgaactgctgcacgctccagccaccgtctgcggacctaaaaagagcaccaacctggtgaagaacaagtgcgtgaatttctga

SEQ ID NO: 2 - DNA, 9616 bp, synthetic construct
  source 1..9616: mol_type = other DNA
ataggcggcgcatgagagaagcccagaccaattacctacccaaaatggagaaagttcacgttgacatcgaggaagacagcccattcctcagagctttgcagcggagcttcccgcagtttgaggtagaagccaagcaggtcactgataatgaccatgctaatgccagagcgttttcgcatctggcttcaaaactgatcgaaacggaggtggacccatccgacacgatccttgacattggaagtgcgcccgcccgcagaatgtattctaagcacaagtatcattgtatctgtccgatgagatgtgcggaagatccggacagattgtataagtatgcaactaagctgaagaaaaactgtaaggaaataactgataaggaattggacaagaaaatgaaggagctcgccgccgtcatgagcgaccctgacctggaaactgagactatgtgcctccacgacgacgagtcgtgtcgctacgaagggcaagtcgctgtttaccaggatgtatacgcggttgacggaccgacaagtctctatcaccaagccaataagggagttagagtcgcctactggataggctttgacaccaccccttttatgtttaagaacttggctggagcatatccatcatactctaccaactgggccgacgaaaccgtgttaacggctcgtaacataggcctatgcagctctgacgttatggagcggtcacgtagagggatgtccattcttagaaagaagtatttgaaaccatccaacaatgttctattctctgttggctcgaccatctaccacgagaagagggacttactgaggagctggcacctgccgtctgtatttcacttacgtggcaagcaaaattacacatgtcggtgtgagactatagttagttgcgacgggtacgtcgttaaaagaatagctatcagtccaggcctgtatgggaagccttcaggctatgctgctacgatgcaccgcgagggattcttgtgctgcaaagtgacagacacattgaacggggagagggtctcttttcccgtgtgcacgtatgtgccagctacattgtgtgaccaaatgactggcatactggcaacagatgtcagtgcggacgacgcgcaaaaactgctggttgggctcaaccagcgtatagtcgtcaacggtcgcacccagagaaacaccaataccatgaaaaattaccttttgcccgtagtggcccaggcatttgctaggtgggcaaaggaatataaggaagatcaagaagatgaaaggccactaggactacgagatagacagttagtcatggggtgttgttgggcttttagaaggcacaagataacatctatttataagcgcccggatacccaaaccatcatcaaagtgaacagcgatttccactcattcgtgctgcccaggataggcagtaacacattggagatcgggctgagaacaagaatcaggaaaatgttagaggagcacaaggagccgtcacctctcattaccgccgaggacgtacaagaagctaagtgcgcagccgatgaggctaaggaggtgcgtgaagccgaggagttgcgcgcagctctaccacctttggcagctgatgttgaggagcccactctggaagccgatgtcgacttgatgttacaagaggctggggccggctcagtggagacacctcgtggcttgataaaggttaccagctacgatggcgaggacaagatcggctcttacgctgtgctttctccgcaggctgtactcaagagtgaaaaattatcttgcatccaccctctcgctgaacaagtcatagtgataacacactctggccgaaaagggcgttatgccgtggaaccataccatggtaaagtagtggtgccagagggacatgcaatacccgtccaggactttcaagctctgagtgaaagtgccaccattgtgtacaacgaacgtgagttcgtaaacaggtacctgcaccatattgccacacatggaggagcgctgaacactgatgaagaatattacaaaactgtcaagcccagcgagcacgacggcgaatacctgtacgacatcgacaggaaacagtgcgtcaagaaagaactagtcactgggctagggctcacaggcgagctggtggatcctcccttccatgaattcgcctacgagagtctgagaacacgaccagccgctccttaccaagtaccaaccataggggtgtatggcgtgccaggatcaggcaagtctggcatcattaaaagcgcagtcaccaaaaaagatctagtggtgagcgccaagaaagaaaactgtgcagaaattataagggacgtcaagaaaatgaaagggctggacgtcaatgccagaactgtggactcagtgctcttgaatggatgcaaacaccccgtagagaccctgtatattgacgaagcttttgcttgtcatgcaggtactctcagagcgctcatagccattataagacctaaaaaggcagtgctctgcggggatcccaaacagtgcggtttttttaacatgatgtgcctgaaagtgcattttaaccacgagatttgcacacaagtcttccacaaaagcatctctcgccgttgcactaaatctgtgacttcggtcgtctcaaccttgttttacgacaaaaaaatgagaacgacgaatccgaaagagactaagattgtgattgacactaccggcagtaccaaacctaagcaggacgatctcattctcacttgtttcagagggtgggtgaagcagttgcaaatagattacaaaggcaacgaaataatgacggcagctgcctctcaagggctgacccgtaaaggtgtgtatgccgttcggtacaaggtgaatgaaaatcctctgtacgcacccacctcagaacatgtgaacgtcctactgacccgcacggaggaccgcatcgtgtggaaaacactagccggcgacccatggataaaaacactgactgccaagtaccctgggaatttcactgccacgatagaggagtggcaagcagagcatgatgccatcatgaggcacatcttggagagaccggaccctaccgacgtcttccagaataaggcaaacgtgtgttgggccaaggctttagtgccggtgctgaagaccgctggcatagacatgaccactgaacaatggaacactgtggattattttgaaacggacaaagctcactcagcagagatagtattgaaccaactatgcgtgaggttctttggactcgatctggactccggtctattttctgcacccactgttccgttatccattaggaataatcactgggataactccccgtcgcctaacatgtacgggctgaataaagaagtggtccgtcagctctctcgcaggtacccacaactgcctcgggcagttgccactggaagagtctatgacatgaacactggtacactgcgcaattatgatccgcgcataaacctagtacctgtaaacagaagactgcctcatgctttagtcctccaccataatgaacacccacagagtgacttttcttcattcgtcagcaaattgaagggcagaactgtcctggtggtcggggaaaagttgtccgtcccaggcaaaatggttgactggttgtcagaccggcctgaggctaccttcagagctcggctggatttaggcatcccaggtgatgtgcccaaatatgacataatatttgttaatgtgaggaccccatataaataccatcactatcagcagtgtgaagaccatgccattaagcttagcatgttgaccaagaaagcttgtctgcatctgaatcccggcggaacctgtgtcagcataggttatggttacgctgacagggccagcgaaagcatcattggtgctatagcgcggcagttcaagttttcccgggtatgcaaaccgaaatcctcacttgaagagacggaagttctgtttgtattcattgggtacgatcgcaaggcccgtacgcacaatccttacaagctttcatcaaccttgaccaacatttatacaggttccagactccacgaagccggatgtgcaccctcatatcatgtggtgcgaggggatattgccacggccaccgaaggagtgattataaatgctgctaacagcaaaggacaacctggcggaggggtgtgcggagcgctgtataagaaattcccggaaagcttcgatttacagccgatcgaagtaggaaaagcgcgactggtcaaaggtgcagctaaacatatcattcatgccgtaggaccaaacttcaacaaagtttcggaggttgaaggtgacaaacagttggcagaggcttatgagtccatcgctaagattgtcaacgataacaattacaagtcagtagcgattccactgttgtccaccggcatcttttccgggaacaaagatcgactaacccaatcattgaaccatttgctgacagctttagacaccactgatgcagatgtagccatatactgcagggacaagaaatgggaaatgactctcaaggaagcagtggctaggagagaagcagtggaggagatatgcatatccgacgactcttcagtgacagaacctgatgcagagctggtgagggtgcatccgaagagttctttggctggaaggaagggctacagcacaagcgatggcaaaactttctcatatttggaagggaccaagtttcaccaggcggccaaggatatagcagaaattaatgccatgtggcccgttgcaacggaggccaatgagcaggtatgcatgtatatcctcggagaaagcatgagcagtattaggtcgaaatgccccgtcgaagagtcggaagcctccacaccacctagcacgctgccttgcttgtgcatccatgccatgactccagaaagagtacagcgcctaaaagcctcacgtccagaacaaattactgtgtgctcatcctttccattgccgaagtatagaatcactggtgtgcagaagatccaatgctcccagcctatattgttctcaccgaaagtgcctgcgtatattcatccaaggaagtatctcgtggaaacaccaccggtagacgagactccggagccatcggcagagaaccaatccacagaggggacacctgaacaaccaccacttataaccgaggatgagaccaggactagaacgcctgagccgatcatcatcgaagaggaagaagaggatagcataagtttgctgtcagatggcccgacccaccaggtgctgcaagtcgaggcagacattcacgggccgccctctgtatctagctcatcctggtccattcctcatgcatccgactttgatgtggacagtttatccatacttgacaccctggagggagctagcgtgaccagcggggcaacgtcagccgagactaactcttacttcgcaaagagtatggagtttctggcgcgaccggtgcctgcgcctcgaacagtattcaggaaccctccacatcccgctccgcgcacaagaacaccgtcacttgcacccagcagggcctgctcgagaaccagcctagtttccaccccgccaggcgtgaatagggtgatcactagagaggagctcgaggcgcttaccccgtcacgcactcctagcaggtcggtctcgagaaccagcctggtctccaacccgccaggcgtaaatagggtgattacaagagaggagtttgaggcgttcgtagcacaacaacaatgacggtttgatgcgggtgcatacatcttttcctccgacaccggtcaagggcatttacaacaaaaatcagtaaggcaaacggtgctatccgaagtggtgttggagaggaccgaattggagatttcgtatgccccgcgcctcgaccaagaaaaagaagaattactacgcaagaaattacagttaaatcccacacctgctaacagaagcagataccagtccaggaaggtggagaacatgaaagccataacagctagacgtattctgcaaggcctagggcattatttgaaggcagaaggaaaagtggagtgctaccgaaccctgcatcctgttcctttgtattcatctagtgtgaaccgtgccttttcaagccccaaggtcgcagtggaagcctgtaacgccatgttgaaagagaactttccgactgtggcttcttactgtattattccagagtacgatgcctatttggacatggttgacggagcttcatgctgcttagacactgccagtttttgccctgcaaagctgcgcagctttccaaagaaacactcctatttggaacccacaatacgatcggcagtgccttcagcgatccagaacacgctccagaacgtcctggcagctgccacaaaaagaaattgcaatgtcacgcaaatgagagaattgcccgtattggattcggcggcctttaatgtggaatgcttcaagaaatatgcgtgtaataatgaatattgggaaacgtttaaagaaaaccccatcaggcttactgaagaaaacgtggtaaattacattaccaaattaaaaggaccaaaagctgctgctctttttgcgaagacacataatttgaatatgttgcaggacataccaatggacaggtttgtaatggacttaaagagagacgtgaaagtgactccaggaacaaaacatactgaagaacggcccaaggtacaggtgatccaggctgccgatccgctagcaacagcgtatctgtgcggaatccaccgagagctggttaggagattaaatgcggtcctgcttccgaacattcatacactgtttgatatgtcggctgaagactttgacgctattatagccgagcacttccagcctggggattgtgttctggaaactgacatcgcgtcgtttgataaaagtgaggacgacgccatggctctgaccgcgttaatgattctggaagacttaggtgtggacgcagagctgttgacgctgattgaggcggctttcggcgaaatttcatcaatacatttgcccactaaaactaaatttaaattcggagccatgatgaaatctggaatgttcctcacactgtttgtgaacacagtcattaacattgtaatcgcaagcagagtgttgagagaacggctaaccggatcaccatgtgcagcattcattggagatgacaatatcgtgaaaggagtcaaatcggacaaattaatggcagacaggtgcgccacctggttgaatatggaagtcaagattatagatgctgtggtgggcgagaaagcgccttatttctgtggagggtttattttgtgtgactccgtgaccggcacagcgtgccgtgtggcagaccccctaaaaaggctgtttaagcttggcaaacctctggcagcagacgatgaacatgatgatgacaggagaagggcattgcatgaagagtcaacacgctggaaccgagtgggtattctttcagagctgtgcaaggcagtagaatcaaggtatgaaaccgtaggaacttccatcatagttatggccatgactactctagctagcagtgttaaatcattcagctacctgagaggggcccctataactctctacggctaacctgaatggactacgacatagtctagtccgccaagtaaggcgcgcccacccagcggccgcatacagcagcaattggcaagctgcttacatagaactcgcggcgattggcatgccgccttaaaatttttattttatttttcttttcttttccgaatcggattttgtttttaatatttcaaaaaaaaaaaaaaaaaaaaaaaaaaaaaaaaaaaaaaaaagaagagctagggataacagggtaattgagcaaaaggccagcaaaaggccaggaaccgtaaaaaggccgcgttgctggcgtttttccataggctccgcccccctgacgagcatcacaaaaatcgacgctcaagtcagaggtggcgaaacccgacaggactataaagataccaggcgtttccccctggaagctccctcgtgcgctctcctgttccgaccctgccgcttaccggatacctgtccgcctttctcccttcgggaagcgtggcgctttctcatagctcacgctgtaggtatctcagttcggtgtaggtcgttcgctccaagctgggctgtgtgcacgaaccccccgttcagcccgaccgctgcgccttatccggtaactatcgtcttgagtccaacccggtaagacacgacttatcgccactggcagcagccactggtaacaggattagcagagcgaggtatgtaggcggtgctacagagttcttgaagtggtggcctaactacggctacactagaagaacagtatttggtatctgcgctctgctgaagccagttaccttcggaaaaagagttggtagctcttgatccggcaaacaaaccaccgctggtagcggtggtttttttgtttgcaagcagcagattacgcgcagaaaaaaaggatctcaagaagatcctttgatcttttctacggggtctgacgctcagtggaacgaaaactcacgttaagggattttggtcatgagattatcaaaaaggatcttcacctagatccttttaaattaaaaatgaagttttaaatcaatctaaagtatatatgagtaaacttggtctgacagttaccaatgcttaatcagtgaggcacctatctcagcgatctgtctatttcgttcatccatagttgcctgactccccgtcgtgtagataactacgatacgggagggcttaccatctggccccagtgctgcaatgataccgcgagacccacgctcaccggctccagatttatcagcaataaaccagccagccggaagggccgagcgcagaagtggtcctgcaactttatccgcctccatccagtctattaattgttgccgggaagctagagtaagtagttcgccagttaatagtttgcgcaacgttgttgccattgctacaggcatcgtggtgtcacgctcgtcgtttggtatggcttcattcagctccggttcccaacgatcaaggcgagttacatgatcccccatgttgtgcaaaaaagcggttagctccttcggtcctccgatcgttgtcagaagtaagttggccgcagtgttatcactcatggttatggcagcactgcataattctcttactgtcatgccatccgtaagatgcttttctgtgactggtgagtactcaaccaagtcattctgagaatagtgtatgcggcgaccgagttgctcttgcccggcgtcaatacgggataataccgcgccacatagcagaactttaaaagtgctcatcattggaaaacgttcttcggggcgaaaactctcaaggatcttaccgctgttgagatccagttcgatgtaacccactcgtgcacccaactgatcttcagcatcttttactttcaccagcgtttctgggtgagcaaaaacaggaaggcaaaatgccgcaaaaaagggaataagggcgacacggaaatgttgaatactcatactcttcctttttcaatattattgaagcatttatcagggttattgtctcatgagcggatacatatttgaatgtatttagaaaaataaacaaataggggttccgcgcacatttccccgaaaagtgccacctgacgttagggataacagggtaattaatacgactcactatag

SEQ ID NO: 3 - RNA, 10366 nt, synthetic construct
  source 1..10366: mol_type = other RNA
ataggcggcgcatgagagaagcccagaccaattacctacccaaaatggagaaagttcacgttgacatcgaggaagacagcccattcctcagagctttgcagcggagcttcccgcagtttgaggtagaagccaagcaggtcactgataatgaccatgctaatgccagagcgttttcgcatctggcttcaaaactgatcgaaacggaggtggacccatccgacacgatccttgacattggaagtgcgcccgcccgcagaatgtattctaagcacaagtatcattgtatctgtccgatgagatgtgcggaagatccggacagattgtataagtatgcaactaagctgaagaaaaactgtaaggaaataactgataaggaattggacaagaaaatgaaggagctcgccgccgtcatgagcgaccctgacctggaaactgagactatgtgcctccacgacgacgagtcgtgtcgctacgaagggcaagtcgctgtttaccaggatgtatacgcggttgacggaccgacaagtctctatcaccaagccaataagggagttagagtcgcctactggataggctttgacaccaccccttttatgtttaagaacttggctggagcatatccatcatactctaccaactgggccgacgaaaccgtgttaacggctcgtaacataggcctatgcagctctgacgttatggagcggtcacgtagagggatgtccattcttagaaagaagtatttgaaaccatccaacaatgttctattctctgttggctcgaccatctaccacgagaagagggacttactgaggagctggcacctgccgtctgtatttcacttacgtggcaagcaaaattacacatgtcggtgtgagactatagttagttgcgacgggtacgtcgttaaaagaatagctatcagtccaggcctgtatgggaagccttcaggctatgctgctacgatgcaccgcgagggattcttgtgctgcaaagtgacagacacattgaacggggagagggtctcttttcccgtgtgcacgtatgtgccagctacattgtgtgaccaaatgactggcatactggcaacagatgtcagtgcggacgacgcgcaaaaactgctggttgggctcaaccagcgtatagtcgtcaacggtcgcacccagagaaacaccaataccatgaaaaattaccttttgcccgtagtggcccaggcatttgctaggtgggcaaaggaatataaggaagatcaagaagatgaaaggccactaggactacgagatagacagttagtcatggggtgttgttgggcttttagaaggcacaagataacatctatttataagcgcccggatacccaaaccatcatcaaagtgaacagcgatttccactcattcgtgctgcccaggataggcagtaacacattggagatcgggctgagaacaagaatcaggaaaatgttagaggagcacaaggagccgtcacctctcattaccgccgaggacgtacaagaagctaagtgcgcagccgatgaggctaaggaggtgcgtgaagccgaggagttgcgcgcagctctaccacctttggcagctgatgttgaggagcccactctggaagccgatgtcgacttgatgttacaagaggctggggccggctcagtggagacacctcgtggcttgataaaggttaccagctacgatggcgaggacaagatcggctcttacgctgtgctttctccgcaggctgtactcaagagtgaaaaattatcttgcatccaccctctcgctgaacaagtcatagtgataacacactctggccgaaaagggcgttatgccgtggaaccataccatggtaaagtagtggtgccagagggacatgcaatacccgtccaggactttcaagctctgagtgaaagtgccaccattgtgtacaacgaacgtgagttcgtaaacaggtacctgcaccatattgccacacatggaggagcgctgaacactgatgaagaatattacaaaactgtcaagcccagcgagcacgacggcgaatacctgtacgacatcgacaggaaacagtgcgtcaagaaagaactagtcactgggctagggctcacaggcgagctggtggatcctcccttccatgaattcgcctacgagagtctgagaacacgaccagccgctccttaccaagtaccaaccataggggtgtatggcgtgccaggatcaggcaagtctggcatcattaaaagcgcagtcaccaaaaaagatctagtggtgagcgccaagaaagaaaactgtgcagaaattataagggacgtcaagaaaatgaaagggctggacgtcaatgccagaactgtggactcagtgctcttgaatggatgcaaacaccccgtagagaccctgtatattgacgaagcttttgcttgtcatgcaggtactctcagagcgctcatagccattataagacctaaaaaggcagtgctctgcggggatcccaaacagtgcggtttttttaacatgatgtgcctgaaagtgcattttaaccacgagatttgcacacaagtcttccacaaaagcatctctcgccgttgcactaaatctgtgacttcggtcgtctcaaccttgttttacgacaaaaaaatgagaacgacgaatccgaaagagactaagattgtgattgacactaccggcagtaccaaacctaagcaggacgatctcattctcacttgtttcagagggtgggtgaagcagttgcaaatagattacaaaggcaacgaaataatgacggcagctgcctctcaagggctgacccgtaaaggtgtgtatgccgttcggtacaaggtgaatgaaaatcctctgtacgcacccacctcagaacatgtgaacgtcctactgacccgcacggaggaccgcatcgtgtggaaaacactagccggcgacccatggataaaaacactgactgccaagtaccctgggaatttcactgccacgatagaggagtggcaagcagagcatgatgccatcatgaggcacatcttggagagaccggaccctaccgacgtcttccagaataaggcaaacgtgtgttgggccaaggctttagtgccggtgctgaagaccgctggcatagacatgaccactgaacaatggaacactgtggattattttgaaacggacaaagctcactcagcagagatagtattgaaccaactatgcgtgaggttctttggactcgatctggactccggtctattttctgcacccactgttccgttatccattaggaataatcactgggataactccccgtcgcctaacatgtacgggctgaataaagaagtggtccgtcagctctctcgcaggtacccacaactgcctcgggcagttgccactggaagagtctatgacatgaacactggtacactgcgcaattatgatccgcgcataaacctagtacctgtaaacagaagactgcctcatgctttagtcctccaccataatgaacacccacagagtgacttttcttcattcgtcagcaaattgaagggcagaactgtcctggtggtcggggaaaagttgtccgtcccaggcaaaatggttgactggttgtcagaccggcctgaggctaccttcagagctcggctggatttaggcatcccaggtgatgtgcccaaatatgacataatatttgttaatgtgaggaccccatataaataccatcactatcagcagtgtgaagaccatgccattaagcttagcatgttgaccaagaaagcttgtctgcatctgaatcccggcggaacctgtgtcagcataggttatggttacgctgacagggccagcgaaagcatcattggtgctatagcgcggcagttcaagttttcccgggtatgcaaaccgaaatcctcacttgaagagacggaagttctgtttgtattcattgggtacgatcgcaaggcccgtacgcacaatccttacaagctttcatcaaccttgaccaacatttatacaggttccagactccacgaagccggatgtgcaccctcatatcatgtggtgcgaggggatattgccacggccaccgaaggagtgattataaatgctgctaacagcaaaggacaacctggcggaggggtgtgcggagcgctgtataagaaattcccggaaagcttcgatttacagccgatcgaagtaggaaaagcgcgactggtcaaaggtgcagctaaacatatcattcatgccgtaggaccaaacttcaacaaagtttcggaggttgaaggtgacaaacagttggcagaggcttatgagtccatcgctaagattgtcaacgataacaattacaagtcagtagcgattccactgttgtccaccggcatcttttccgggaacaaagatcgactaacccaatcattgaaccatttgctgacagctttagacaccactgatgcagatgtagccatatactgcagggacaagaaatgggaaatgactctcaaggaagcagtggctaggagagaagcagtggaggagatatgcatatccgacgactcttcagtgacagaacctgatgcagagctggtgagggtgcatccgaagagttctttggctggaaggaagggctacagcacaagcgatggcaaaactttctcatatttggaagggaccaagtttcaccaggcggccaaggatatagcagaaattaatgccatgtggcccgttgcaacggaggccaatgagcaggtatgcatgtatatcctcggagaaagcatgagcagtattaggtcgaaatgccccgtcgaagagtcggaagcctccacaccacctagcacgctgccttgcttgtgcatccatgccatgactccagaaagagtacagcgcctaaaagcctcacgtccagaacaaattactgtgtgctcatcctttccattgccgaagtatagaatcactggtgtgcagaagatccaatgctcccagcctatattgttctcaccgaaagtgcctgcgtatattcatccaaggaagtatctcgtggaaacaccaccggtagacgagactccggagccatcggcagagaaccaatccacagaggggacacctgaacaaccaccacttataaccgaggatgagaccaggactagaacgcctgagccgatcatcatcgaagaggaagaagaggatagcataagtttgctgtcagatggcccgacccaccaggtgctgcaagtcgaggcagacattcacgggccgccctctgtatctagctcatcctggtccattcctcatgcatccgactttgatgtggacagtttatccatacttgacaccctggagggagctagcgtgaccagcggggcaacgtcagccgagactaactcttacttcgcaaagagtatggagtttctggcgcgaccggtgcctgcgcctcgaacagtattcaggaaccctccacatcccgctccgcgcacaagaacaccgtcacttgcacccagcagggcctgctcgagaaccagcctagtttccaccccgccaggcgtgaatagggtgatcactagagaggagctcgaggcgcttaccccgtcacgcactcctagcaggtcggtctcgagaaccagcctggtctccaacccgccaggcgtaaatagggtgattacaagagaggagtttgaggcgttcgtagcacaacaacaatgacggtttgatgcgggtgcatacatcttttcctccgacaccggtcaagggcatttacaacaaaaatcagtaaggcaaacggtgctatccgaagtggtgttggagaggaccgaattggagatttcgtatgccccgcgcctcgaccaagaaaaagaagaattactacgcaagaaattacagttaaatcccacacctgctaacagaagcagataccagtccaggaaggtggagaacatgaaagccataacagctagacgtattctgcaaggcctagggcattatttgaaggcagaaggaaaagtggagtgctaccgaaccctgcatcctgttcctttgtattcatctagtgtgaaccgtgccttttcaagccccaaggtcgcagtggaagcctgtaacgccatgttgaaagagaactttccgactgtggcttcttactgtattattccagagtacgatgcctatttggacatggttgacggagcttcatgctgcttagacactgccagtttttgccctgcaaagctgcgcagctttccaaagaaacactcctatttggaacccacaatacgatcggcagtgccttcagcgatccagaacacgctccagaacgtcctggcagctgccacaaaaagaaattgcaatgtcacgcaaatgagagaattgcccgtattggattcggcggcctttaatgtggaatgcttcaagaaatatgcgtgtaataatgaatattgggaaacgtttaaagaaaaccccatcaggcttactgaagaaaacgtggtaaattacattaccaaattaaaaggaccaaaagctgctgctctttttgcgaagacacataatttgaatatgttgcaggacataccaatggacaggtttgtaatggacttaaagagagacgtgaaagtgactccaggaacaaaacatactgaagaacggcccaaggtacaggtgatccaggctgccgatccgctagcaacagcgtatctgtgcggaatccaccgagagctggttaggagattaaatgcggtcctgcttccgaacattcatacactgtttgatatgtcggctgaagactttgacgctattatagccgagcacttccagcctggggattgtgttctggaaactgacatcgcgtcgtttgataaaagtgaggacgacgccatggctctgaccgcgttaatgattctggaagacttaggtgtggacgcagagctgttgacgctgattgaggcggctttcggcgaaatttcatcaatacatttgcccactaaaactaaatttaaattcggagccatgatgaaatctggaatgttcctcacactgtttgtgaacacagtcattaacattgtaatcgcaagcagagtgttgagagaacggctaaccggatcaccatgtgcagcattcattggagatgacaatatcgtgaaaggagtcaaatcggacaaattaatggcagacaggtgcgccacctggttgaatatggaagtcaagattatagatgctgtggtgggcgagaaagcgccttatttctgtggagggtttattttgtgtgactccgtgaccggcacagcgtgccgtgtggcagaccccctaaaaaggctgtttaagcttggcaaacctctggcagcagacgatgaacatgatgatgacaggagaagggcattgcatgaagagtcaacacgctggaaccgagtgggtattctttcagagctgtgcaaggcagtagaatcaaggtatgaaaccgtaggaacttccatcatagttatggccatgactactctagctagcagtgttaaatcattcagctacctgagaggggcccctataactctctacggctaacctgaatggactacgacatagtctagtccgccaagatgcccatggggtctctgcaaccgctggccaccttgtacctgctggggatgctggtcgcttccgtgctagcctctagacgggtgcagcctacagagagcatcgtgcggttccctaacatcaccaacctctgccccttcggcgaggtgttcaacgccaccagattcgccagcgtctacgcctggaaccggaagcggatcagcaattgcgtggccgactacagcgtgctgtacaacagcgccagcttcagcaccttcaagtgctacggcgtgtcccctaccaagctgaacgatctgtgcttcaccaacgtgtacgccgacagcttcgtgatcaggggcgacgaagtgcgacagatcgccccaggacagacaggaaagatcgccgattacaactacaagctgcccgacgacttcaccggttgcgtgatcgcttggaacagcaacaacctggacagcaaggtcggcggcaactacaactacctgtaccggctgttccggaagtccaacctgaagcccttcgagcgggacatcagcacagagatctaccaggccggcagcacaccttgtaacggcgtggagggcttcaactgctacttccctctgcagagctacggcttccagcctacaaacggcgtgggataccagccttacagggtggtggtgctgagcttcgaactgctgcacgctccagccaccgtctgcggacctaaaaagagcaccaacctggtgaagaacaagtgcgtgaatttctgataaggcgcgcccacccagcggccgcatacagcagcaattggcaagctgcttacatagaactcgcggcgattggcatgccgccttaaaatttttattttatttttcttttcttttccgaatcggattttgtttttaatatttcaaaaaaaaaaaaaaaaaaaaaaaaaaaaaaaaaaaaaaaaagaagagctagggataacagggtaattgagcaaaaggccagcaaaaggccaggaaccgtaaaaaggccgcgttgctggcgtttttccataggctccgcccccctgacgagcatcacaaaaatcgacgctcaagtcagaggtggcgaaacccgacaggactataaagataccaggcgtttccccctggaagctccctcgtgcgctctcctgttccgaccctgccgcttaccggatacctgtccgcctttctcccttcgggaagcgtggcgctttctcatagctcacgctgtaggtatctcagttcggtgtaggtcgttcgctccaagctgggctgtgtgcacgaaccccccgttcagcccgaccgctgcgccttatccggtaactatcgtcttgagtccaacccggtaagacacgacttatcgccactggcagcagccactggtaacaggattagcagagcgaggtatgtaggcggtgctacagagttcttgaagtggtggcctaactacggctacactagaagaacagtatttggtatctgcgctctgctgaagccagttaccttcggaaaaagagttggtagctcttgatccggcaaacaaaccaccgctggtagcggtggtttttttgtttgcaagcagcagattacgcgcagaaaaaaaggatctcaagaagatcctttgatcttttctacggggtctgacgctcagtggaacgaaaactcacgttaagggattttggtcatgagattatcaaaaaggatcttcacctagatccttttaaattaaaaatgaagttttaaatcaatctaaagtatatatgagtaaacttggtctgacagttaccaatgcttaatcagtgaggcacctatctcagcgatctgtctatttcgttcatccatagttgcctgactccccgtcgtgtagataactacgatacgggagggcttaccatctggccccagtgctgcaatgataccgcgagacccacgctcaccggctccagatttatcagcaataaaccagccagccggaagggccgagcgcagaagtggtcctgcaactttatccgcctccatccagtctattaattgttgccgggaagctagagtaagtagttcgccagttaatagtttgcgcaacgttgttgccattgctacaggcatcgtggtgtcacgctcgtcgtttggtatggcttcattcagctccggttcccaacgatcaaggcgagttacatgatcccccatgttgtgcaaaaaagcggttagctccttcggtcctccgatcgttgtcagaagtaagttggccgcagtgttatcactcatggttatggcagcactgcataattctcttactgtcatgccatccgtaagatgcttttctgtgactggtgagtactcaaccaagtcattctgagaatagtgtatgcggcgaccgagttgctcttgcccggcgtcaatacgggataataccgcgccacatagcagaactttaaaagtgctcatcattggaaaacgttcttcggggcgaaaactctcaaggatcttaccgctgttgagatccagttcgatgtaacccactcgtgcacccaactgatcttcagcatcttttactttcaccagcgtttctgggtgagcaaaaacaggaaggcaaaatgccgcaaaaaagggaataagggcgacacggaaatgttgaatactcatactcttcctttttcaatattattgaagcatttatcagggttattgtctcatgagcggatacatatttgaatgtatttagaaaaataaacaaataggggttccgcgcacatttccccgaaaagtgccacctgacgttagggataacagggtaattaatacgactcactatag